European Patent Specification EP 3 283 104 B1, published December 11, 2024. Title: Arenaviren zur Anwendung bei der Therapie von Karzinomen oder Sarkomen sowie Verfahren zur Herstellung von Arenaviren mit einer verbesserten immuntherapeutischen Wirkung gegenüber Karzinomen oder Sarkomen. Applicant: Lang Karl Sebastian. The sequence listing filed with the application follows.

SEQUENCE LISTING (6 sequences)

SEQ ID NO: 1 - RNA, 3413 nt, Junin virus
  Junin virus strain Candid-1 segment S - AY746353 - viruses; ssrna negative-strand viruses; arenaviridae; arenavirus; new world arenaviruses
gtgcagtaaggggatcctaggcgattttggttacgctataattgtaactgttttctgtttggacaacatcaaaaacatccattgcacaatggggcagttcattagcttcatgcaagaaataccaacctttttgcaggaggctctgaacattgctcttgttgcagtcagtctcattgccatcattaagggtatagtgaacttgtacaaaagtggtttattccaattctttgtattcctagcgcttgcaggaagatcctgcacagaagaagctttcaaaatcggactgcacactgagttccagactgtgtccttctcaatggtgggtctcttttccaacaatccacatgacctacctttgttgtgtaccttaaacaagagccatctttacattaaggggggcaatgcttcatttcagatcagctttgatgatattgcagtattgttgccacagtatgatgttataatacaacatccagcagatatgagctggtgttccaaaagtgatgatcaaatttggttgtctcagtggttcatgaatgctgtggggcatgattggcatctagacccaccatttctgtgtaggaaccgtgcaaagacagaaggcttcatctttcaagtcaacacctccaagactggtgtcaatggaaattatgctaagaagtttaagactggcatgcatcatttatatagagaatatcctgacccttgcttgaatggcaaactgtgcttaatgaaggcacaacctaccagttggcctctccaatgtccactcgaccacgttaacacattacacttccttacaagaggtaaaaacattcaacttccaaggaggtccttgaaagcattcttctcctggtctttgacagactcatccggcaaggatacccctggaggctattgtctagaagagtggatgctcgtagcagccaaaatgaagtgttttggcaatactgctgtagcaaaatgcaatttgaatcatgactctgaattctgtgacatgttgaggctctttgattacaacaaaaatgctatcaaaaccctaaatgatgaaactaagaaacaagtaaatctgatggggcagacaatcaatgccctgatatctgacaatttattgatgaaaaacaaaattagggaactgatgagtgtcccttactgcaattacacaaaattttggtatgtcaaccacacactttcaggacaacactcattaccaaggtgctggttaataaaaaacaacagctatttgaacatctctgacttccgtaatgactggatattagaaagtgacttcttaatttctgaaatgctaagcaaagagtattcggacaggcagggtaaaactcctttgactttagttgacatctgtatttggagcacagtattcttcacagcgtcactcttccttcacttggtgggtataccctcccacagacacatcaggggcgaagcatgccctttgccacacaggttgaacagcttgggtggttgcagatgtggtaagtaccccaatctaaagaaaccaacagtttggcgtagaggacactaagacctcctgagggtccccaccagcccgggcactgcccgggctggtgtggccccccagtccgcggcctggccgcggactggggaggcactgcttacagtgcataggctgccttcgggaggaacagcaagctcggtggtaatagaggtgtaggttcctcctcatagagcttcccatctagcactgactgaaacattatgcagtctagcagagcacagtgtggttcactggaggccaacttgaagggagtatccttttccctctttttcttattgacaaccactccattgtgatatttgcataagtgaccatatttctcccagacctgttgatcaaactgcctggcttgttcagatgtgagcttaacatcaaccagtttaagatctcttcttccatggaggtcaaacaacttcctgatgtcatcggatccttgagtagtcacaaccatgtctggaggcagcaagccgatcacgtaactaagaactcctggcattgcatcttctatgtccttcattaagatgccgtgagagtgtctgctaccatttttaaaccctttctcatcatgtggttttctgaagcagtgaatgtactgcttacctgcaggttggaataatgccatctcaacagggtcagtggctggtccttcaatgtcgagccaaagggtgttggtggggtcgagtttccccactgcctctctgatgacagcttcttgtatctctgtcaagttagccaatctcaaattctgaccgtttttttccggctgtctaggaccagcaactggtttccttgtcagatcaatacttgtgttgtcccatgacctgcctgtgatttgtgatctagaaccaatataaggccaaccatcgccagaaagacaaagtttgtacaaaaggttttcataaggatttctattgcctggtttctcatcaataaacatgccttctcttcgtttaacctgaatggttgattttatgagggaagagaagttttctggggtgactctgattgtttccaacatgtttccaccatcaagaatagatgctccagcctttactgcagctgaaagactgaagttgtaaccagaaatattgatggagctttcatctttagtcacaatctgaaggcagtcatgttcctgagtcagtctgtcaaggtcacttaagtttggatacttcacagtgtatagaagcccaagtgaggttaaagcttgtatgacactgttcattgtctcacctccttgaacagtcatgcatgcaattgtcaatgcaggaacagagccaaactgattgtttagctttgaagggtctttaacatcccatatcctcaccacaccatttcccccagtcccttgctgttgaaatcccagtgttctcaatatctctgatcttttagcaagttgtgactgggacaagttacccatgtaaaccccctgagagcctgtctctgctcttcttatcttgttttttaatttctcaaggtcagacgccaactccatcagttcatccctccccagatctcccaccttgaaaactgtgtttcgttgaacactcctcatggacatgagtctgtcaacctctttattcaggtccctcaacttgttgaggtcttcttccccctttttagtctttctgagtgcccgctgcacctgtgccacttggttgaagtcgatgctgtcagcaattagcttggcgtccttcaaaacatctgacttgacagtctgagtgaattggctcaaacctctccttaaggactgagtccatctaaagcttggaacctccttggagtgtgccatgccagaagttctggtgattttgatctagaatagagttgctcagtgaaagtgttagacactatgcctaggatccactgtgcg

SEQ ID NO: 2 - RNA, 7114 nt, Junin virus
  Junin virus strain Candid #1 segment L - AY819707 - viruses; ssrna negative-strand viruses; arenaviridae; arenavirus; new world arenaviruses
cgcacagtggatcctaggcgtaacttcatcattaaaatctcagattctgctctgagtgtgacttactgcgaagaggcagacaaatgggcaactgcaacggggcatccaagtctaaccagccagactcctcaagagccacacagccagccgcagaatttaggagggtagctcacagcagtctatatggtagatataactgtaagtgctgctggtttgctgataccaatttgataacctgtaatgatcactacctttgtttaaggtgccatcagggtatgttaaggaattcagatctctgcaatatctgctggaagcccctgcccaccacaatcacagtaccggtggagccaacagcaccaccaccataggcagactgcacagggtcagacccgaccccccggggggcccccatggggaccccccgtgggggaaccccgggggtgatgcgccattagtcaatgtctttgatctcgactttgtgcttcagtggcctgcatgtcacccctttcaatctgaactgcccttggggatctgatatcagcaggtcatttaaagatctgctgaatgccaccttgaaatttgagaattccaaccagtcaccaaatttatcaagtgaacggatcaactgctctttgtgtagatcataaacgaggacaaagtcctcttgctgaaataatattgtttgtgatgttgtttttagataaggccatagttggcttaataaggtttccacactatcaatgtcctctagtgctccaattgccttgactatgacatccccagacaactcaactctatatgttgacaacctttcattacctctgtaaaagataccctctttcaagacaagaggttctcctgggttatctggcccaatgaggtcatatgcatacttgttacttagttcagaataaaagtcaccaaagttgaacttaacatggctcagaatattgtcatcatttgtcgcagcgtagcctgcatcaataaacaagccagctaggtcaaagctctcatggcctgtgaacaatggtaggctagcgataaccagtgcaccatccaacaatgagtggcttccctcagacccagaaacacattgactcattgcatccacattcagctctaattcaggggtaccgacatcatccactcctagtgaactgacaatggtgtaactgtacaccatctttcttctaagtttaaattttgtcgaaactcgtgtgtgttctacttgaatgatcaattttagtttcacagcttcttggcaagcaacattgcgcaacacagtgtgcaggtccatcatgtcttcctgaggcaacaaggagatgttgtcaacagagacaccctcaaggaaaaccttgatattatcaaagctagaaactacataacccattgcaatgtcttcaacaaacattgctcttgatactttattattcctaactgacaaggtaaaatctgtgagttcagctagatctacttgactgtcatcttctagatctagaacttcattgaaccaaaagaaggatttgagacacgatgttgacatgactagtgggtttatcatcgaagataagacaacttgcaccatgaagttcctgcaaacttgctgtgggctgatgccaacttcccaatttgtatactctgactgtctaacatgggctgaagcgcaatcactctgtttcacaatataaacattattatctcttactttcaataagtgacttataatccctaagttttcattcatcatgtctagagccacacagacatctagaaacttgagtcttccactatccaaagatctgttcacttgaagatcattcataaagggtgccaaatgttcttcaaatagtttggggtaatttcttcgtatagaatgcaatacatggttcatgcctaattggtcttctatctgtcgtactgctttgggtttaacagcccagaagaaattcttattacataagaccagaggggcctgtggactcttaatagcaaaaaacacccactcccctaactcacaggcatttgtcagcaccaaagagaagtaatcccacaaaattggtttagaaaattggttaacttctttaagtgatttttgacagtaaataactttaggctttctctcacaaattccacaaagacatggcattattcgagtaaatatgtcctttatatacagaaatccgcctttaccatccctaacacacttactccccatactcttacaaaacccaatgaagcctgaggcaacagaagactgaaatgcagatttgttgattgactctgccaagatcttcttcacgccttttgtgaaatttcttgacagcctggactgtattgtccttatcaatgttggcatctcttctttctctaacactcttcgacttgtcatgagtttggtcctcaagaccaacctcaagtccccaaagctcgctaaattgacccatctgtagtctagagtttgtctgatttcatcttcactacacccggcatattgcaggaatccggataaagcctcatcccctcccctgcttatcaagttgataaggttttcctcaaagattttgcctctcttaatgtcattgaacactttcctcgcgcagttccttataaacattgtctccttatcatcagaaaaaatagcttcaattttcctctgtagacggtaccctctagacccatcaacccagtctttgacatcttgttcttcaatagctccaaacggagtctctctgtatccagagtatctaatcaattggttgactctaatggaaatctttgacactatatgagtgctaaccccattagcaatacattgatcacaaattgtgtctatggtctctgacagttgtgttggagttttacacttaacgttgtgtagagcagcagacacaaacttggtgagtaaaggagtctcttcacccatgacaaaaaatcttgacttaaactcagcaacaaaagttcctatcacactctttgggctgataaacttgtttaatttagaagataagaattcatggaagcacaccatttccagcagttctgtcctgtcttgaaacttttcatcactaaggcaaggaatttttataaggctaacctggtcatcgctggaggtataagtgacaggtatcacatcatacaataagtcaagtgcataacacagaaattgttcagtaattagcccatataaatctgatgtgttgtgcaagattccctggcccatgtccaagacagacattatatggctggggacctggtcccttgactgcagatactggtgaaaaaactcttcaccaacactagtacagtcacaacccattaaacctaaagatctcttcaatttccctacacagtaggcttctgcaacattaattggaacttcaacgaccttatgaagatgccatttgagaatgttcattactggttcaagattcacctttgttctatctctgggattcttcaattctaatgtgtacaaaaaagaaaggaaaagtgctgggctcatagttggtccccatttggagtggtcatatgaacaggacaagtcaccattgttaacagccattttcatatcacagattgcacgttcgaattccttttctgaattcaagcatgtgtatttcattgaactacccacagcttctgagaagtcttcaactaacctggtcatcagcttagtgttgaggtctcccacatacagttctctatttgagccaacctgctccttataacttagtccaaatttcaagttccctgtatttgagctgatgcttgtgaactctgtaggagagtcgtctgaatagaaacataaattccgtagggctgcatttgtaaaataacttttgtctagcttatcagcaatggcttcagaattgctttccctggtactaagccgaacctcatcctttagtctcagaacttcactggaaaagcccaatctagatctacttctatgctcataactacccaatttctgatcataatgtccttgaattaaaagatacttgaagcattcaaagaattcatcttcttggtaggctattgttgtcaaattttttaataacaaacccaaagggcagatgtcctgcggtgcttcaagaaaataagtcaatttaaatggagatagataaacagcatcacataactctttatacacatcagacctgagcacatctggatcaaaatccttcacctcatgcattgacacctctgctttaatctctctcaacactccaaaaggggcccacaatgactcaagagactctcgctcatcaacagatggattttttgatttcaacttggtgatctcaacttttgtcccctcactattagccatcttggctagtgtcatttgtacgtcatttctaataccctcaaaggcccttacttgatcctctgttaaactctcatacatcactgataattcttcttgattggttctggttcttgaaccggtgctcacaagacctgttagattttttaatattaagtagtccatggaatcaggatcaagattatacctgccttttgttttaaacctctcagccatagtagaaacgcatgttgaaacaagtttctccttatcataaacagaaagaatatttccaagttcgtcgagcttggggattaccacacttttattgcttgacagatccagagctgtgctagtgatgttaggcctgtagggattgcttttcagttcacctgtaactttaagtcttcctctattgaagagagaaatgcagaaggacaaaatctctttacacactcctggaatttgagtatctgaggaagtcttagcctctttggaaaagaatctgtccaatcctcttatcatggtgtcctcttgttccagtgttagactcccacttagaggggggtttacaacaacacaatcaaacttgactttgggctcaataaacttctcaaaacacttgatttgatctgtcaggcgatcaggtgtctctttggttaccaagtgacacagataactaacatttaatagatatttaaaccttcttgcaaagtaaagatctgcatcttccccttcacccaaaattgtctggaaaagttccacagccatcctctgaatcagcacctctgatccagacatgcagtcgacccttaactttgacatcaaatccacatgatggatttgatttgcatatgccatcaagaaatatcttagaccttgtaaaaatgtctggttccttttggaaggggaacagagtacagctaacactaacaatcttaatattggccttgtcattgtcatgagttcgtggctaaaatccaaccagctggtcatttcctcacacatttcaattaacacatcctccgaaaatataggcaggaaaaatctctttggatcacagtaaaaagagccttgttcttccaataccccattgatggatagatagatagaatagcaccttgacttctcacctgttttttggtaaaacaagagaccaaatgtattctttgtcagatgaaatctttgtacataacactctcttagtctaacattcccaaaatatctagaatactctctttcattgattaacaatcgggaggaaaatgatgtcttcatcgagttgaccaatgcaagggaaatggaggacaaaatcctaaataatttcttctgctcaccttccactaagctgctgaatggctgatgtctacagattttctcaaattccttgttaatagtatatctcatcactggtctgtcagaaacaagtgcctgagctaaaatcatcaagctatccatatcagggtgttttattagtttttccagctgtgaccagagatcttgatgagagttcttcaatgttctggaacacgcttgaacccacttggggctggtcatcaatttcttccttattagtttaatcgcctccagaatatctagaagtctgtcattgactaacattaacatttgtccaacaactattcccgcatttcttaaccttacaattgcatcatcatgcgttttgaaaagatcacaaagtaaattgagtaaaactaagtccagaaacagtaaagtgtttctcctggtgttgaaaacttttagacctttcactttgttacacacggaaagggcttgaagataacacctctctacagcatcaatagatatagaattctcatctgactggctttccatgttgacttcatctattggatgcaatgcgatagagtagactacatccatcaacttgtttgcacaaaaagggcagctgggcacatcactgtctttgtggcttcctaataagatcaagtcatttataagcttagacttttgtgaaaatttgaatttccccaactgcttgtcaaaaatctccttcttaaaccaaaaccttaactttatgagttcttctcttatgacagattctctaatgtctcctctaaccccaacaaagagggattcatttaacctctcatcataacccaaagaattctttttcaagcattcgatgttttctaatcccaagctctggttttttgtgttggacaaactatggatcaatcgctggtattcttgttcttcaatattaatctcttgcataaattttgatttctttaggatgtcgatcagcaaccaccgaactctttcaacaacccaatcagcaaggaatctattgctgtagctagatctgccatcaaccacaggaaccaacgtaatccctgcccttagtaggtcggactttaggtttaagagctttgacatgtcactcttccattttctctcaaactcatcaggattgaccctaacaaaggtttccaataggatgagtgttttccctgtgagtttgaagccatccggaatgacttttggaagggtgggacatagtatgccatagtcagacaggatcacatcaacaaacttctgatctgaattgatctgacaggcgtgtgcctcacaggactcaagctctactaaacttgacagaagtttgaacccttccaacaacagagagctggggtgatgttgagataaaaagatgtccctttggtatgctagctcctgtctttctggaaaatgctttctaataaggctttttatttcatttactgattcctccatgctcaagtgccgcctaggatccactgtgcg

SEQ ID NO: 3 - RNA, 3410 nt, Junin mammarenavirus
  Junin virus strain Candid #1 segment S, completesequence.-ACCESSION FJ969442-VERSION FJ969442.1-GI:264665554 - Viruses; ssRNA viruses; ssRNA negative-strand viruses; Arenaviridae; Mammarenavirus.
cgcacagtggatcctaggcgattttggttacgctataattgtaactgttttctgtttggacaacatcaaaaacatccattgcacaatggggcagttcattagcttcatgcaagaaataccaacctttttgcaggaggctctgaacattgctcttgttgcagtcagtctcattgccatcattaagggtgtagtgaacctgtacaaaagtggtttgttccaattctttgtattcctagcactcgcaggaagatcctgcacagaagaagcttttaaaatcggactgcacacagagttccagactgtgtccttctcaatggtgggtctcttttccaacaatccacatgacctgcctctgttgtgtaccttaaacaagagccatctttacattaaggggggcaatgcttcatttcagatcagctttgatgatattgcagtattgttgccacagtatgatgttataatacaacatccagcagatatgagctggtgttccaaaagtgatgatcaaatttggttgtctcagtggttcatgaatgctgtgggacatgattggcatctagacccaccatttctgtgtaggaaccgtgcaaagacagaaggcttcatctttcaagtcaacacctccaagactggtgtcaatggaaattatgctaagaagtttaagactggcatgcatcatttatatagagaatatcctgacccttgcttgaatggcaaactgtgcttaatgaaggcacaacctaccagttggcctctccaatgtccactcgaccacgttaacacattacacttccttacaagaggtaaaaacattcaacttccaaggaggtccttgaaagcattcttctcctggtctttgacagactcatccggcaaggatacccctggaggctattgtctagaagagtggatgctcgttgcagccaaaatgaagtgttttggcaatactgctgtagcaaaatgcaatctgaatcatgactctgaattctgtgacatgctgaggctttttgattacaacaaaaatgctatcaaaaccttaaatgatgaaactaagaaacaagtaaatctgatgggacagacaatcaatgcgctgatatctgacaatttattgatgaaaaacaaaattagggaactgatgagtgtcccttactgcaattacacaaaattttggtatgtcaaccacacactttcaggacaacactcattaccaaggtgctggttaataaaaaacaacagctatttgaacatctctgacttccgtaatgactggatattagaaagtgacttcttaatttctgaaatgctaagcaaagagtattcggacaggcagggtaaaactcctttgactttagttgacatctgtatttggagcacagtattcttcacagcgtcactcttccttcacttggtgggtataccctcccacagacacatcaggggcgaagcatgccctttgccacacaggttgaacagcttgggtggttgcagatgtggtaagtaccccaatctaaagaaaccaacagtttggcgtagaggacactaagacctcctgagggtccccaccagcccgggcactgcccgggctggtgtggccccccagtccgcggcctggccgcggactggggaggcactgcttacagtgcataggctgccttcgggaggaacagcaagctcggtggtaatagaggtgtaggttcctcctcatagagcttcccatctagcactgactgaaacattatgcagtctagcagagcacagtgtggttcactggaggccaacttgaagggagtatccttttccctctttttcttattgacaaccactccattgtgatatttgcataagtgaccatatttctcccagacctgttgatcaaactgcctggcttgttcagatgtgagcttaacatcaaccagtttaagatctcttcttccatggaggtcaaacaacttcctgatgtcatcggatccttgagtagtcacaaccatgtctggaggcagcaagccgatcacgtaactaagaactcctggcattgcatcttctatgtctttcattaagatgccgtgagagtgtctgctaccatttttaaaccctttctcatcatgtggttttctgaagcagtgaatatactgcttacctgcaggctggaacaacgccatctcaacagggtcagtagctggtccttcaatgtcgagccaaagggtattggtggggtcgagtttccccactgcctctctgatgacagcttcttgtatctctgtcaagttagccaatctcaaattctgaccgttcttttccggttgtctaggtccagcaactggtttccttgtcagatcaatacttgtgttgtcccatgacctgcctatgatttgtgatctggaaccaatataaggccaaccatcgccagaaaggcaaagtttgtacagaaggttttcataagggtttctattgcctggtttctcatcaataaacatgccttctcttcgtttaacctgaatggttgattttatgagggaagaaaagttatctggggtgactctgattgtctccaacatatttccaccatcaagaatggatgcaccagcctttactgcagctgaaagactaaagttgtagccagaaatgttgatggagctttcatccttagtcacaatctggaggcagtcatgttcctgagtcaatctgtcaaggtcactcaagtttggatacttcacagtgtatagaagcccaagagaggttaaagcctgtatgacactgttcattgtctcacctccttgaacagtcatgcatgcaattgtcaatgcaggaacagaaccaaactgattgttaagttttgaaggatctttaacatcccataccctcaccacaccatttcccccagttccttgctgttgaaatcccagtgttctcaatatctctgatctcttggccagttgtgattgagacaagttacccatgtaaaccccttgagagcctgtctctgctcttctaatcttgttttttaatttctcaaggtcagacgccaactccatcagttcatccctccccagatctcccaccttgaaaactgtgtttcgttgaacactcctcatggacatgagtctgtcaacctctttattcaggtccctcaacttattgaggtcttcttccccccttttagtctttctgagtgcccgctgcacctgtgcctcttggttgaagtcaatgctgtcagcaattagcttggcatccttcagaacatccgacttgacagtctgagtaaattgactcaaacctctccttaaggactgagtccatctaaagcttggaacctctttggagtgtgccatgccagaagttctggtgattttgatctagaatagagttgctcagtgaaagtgttagacactatgcctaggatccactgtgcg

SEQ ID NO: 4 - RNA, 7114 nt, Junin mammarenavirus; identical to SEQ ID NO: 2
  Junin virus strain Candid #1 segment L, complete sequence.-ACCESSION AY819707-VERSION AY819707.2-GI:227957900-Viruses; ssRNA viruses; ssRNA negative-strand viruses; Arenaviridae; Mammarenavirus.

SEQ ID NO: 5 - RNA, 3377 nt, Lymphocytic choriomeningitis mammarenavirus Viruses (LCMV)
  Lymphocytic choriomeningitis virus clone 13 segment S, complete sequence.ACCESSION DQ361065-VERSION DQ361065.2-GI:116563461.-ssRNA viruses; ssRNA negative-strand viruses; Arenaviridae; Mammarenavirus.
gcgcaccggggatcctaggctttttggattgcgctttcctctagatcaactgggtgtcaggccctatcctacagaaggatgggtcagattgtgacaatgtttgaggctctgcctcacatcatcgatgaggtgatcaacattgtcattattgtgcttatcgtgatcacgggtatcaaggctgtctacaattttgccacctgtgggatattcgcattgatcagtttcctacttctggctggcaggtcctgtggcatgtacggtcttaagggacccgacatttacaaaggagtttaccaatttaagtcagtggagtttgatatgtcacatctgaacctgaccatgcccaacgcatgttcagccaacaactcccaccattacatcagtatggggacttctggactagaattgaccttcaccaatgattccatcatcagtcacaacttttgcaatctgacctctgccttcaacaaaaagacctttgaccacacactcatgagtatagtttcgagcctacacctcagtatcagagggaactccaactataaggcagtatcctgcgacttcaacaatggcataaccatccaatacaacttgacattctcagatgcacaaagtgctcagagccagtgtagaaccttcagaggtagagtcctagatatgtttagaactgccttcggggggaaatacatgaggagtggctggggctggacaggctcagatggcaagaccacctggtgtagccagacgagttaccaatacctgattatacaaaatagaacctgggaaaaccactgcacatatgcaggtccttttgggatgtccaggattctcctttcccaagagaagactaagttcctcactaggagactagcgggcacattcacctggactttgtcagactcttcaggggtggagaatccaggtggttattgcctgaccaaatggatgattcttgctgcagagcttaagtgtttcgggaacacagcagttgcgaaatgcaatgtaaatcatgatgaagaattctgtgacatgctgcgactaattgactacaacaaggctgctttgagtaagttcaaagaggacgtagaatctgccttgcacttattcaaaacaacagtgaattctttgatttcagatcaactactgatgaggaaccacttgagagatctgatgggggtgccatattgcaattactcaaagttttggtacctagaacatgcaaagaccggcgaaactagtgtccccaagtgctggcttgtcaccaatggttcttacttaaatgagacccacttcagtgaccaaatcgaacaggaagccgataacatgattacagagatgttgaggaaggattacataaagaggcaggggagtacccccctagcattgatggaccttctgatgttttccacatctgcatatctagtcagcatcttcctgcaccttgtcaaaataccaacacacaggcacataaaaggtggctcatgtccaaagccacaccgattaaccaacaaaggaatttgtagttgtggtgcatttaaggtgcctggtgtaaaaaccgtctggaaaagacgctgaagaacagcgcctccctgactctccacctcgaaagaggtggagagtcagggaggcccagagggtcttagagtgtcacaacatttgggcctctaaaaattaggtcatgtggcagaatgttgtgaacagttttcagatctgggagccttgctttggaggcgctttcaaaaatgatgcagtccatgagtgcacagtgcggggtgatctctttcttctttttgtcccttactattccagtatgcatcttacacaaccagccatatttgtcccacactttgtcttcatactccctcgaagcttccctggtcatttcaacatcgataagcttaatgtccttcctattctgtgagtccagaagctttctgatgtcatcggagccttgacagcttagaaccatcccctgcggaagagcacctataactgacgaggtcaacccgggttgcgcattgaagaggtcggcaagatccatgccgtgtgagtacttggaatcttgcttgaattgtttttgatcaacgggttccctgtaaaagtgtatgaactgcccgttctgtggttggaaaattgctatttccactggatcattaaatctaccctcaatgtcaatccatgtaggagcgttggggtcaattcctcccatgaggtcttttaaaagcattgtctggctgtagcttaagcccacctgaggtggacctgctgctccaggcgctggcctgggtgaattgactgcaggtttctcgcttgtgagatcaattgttgtgttttcccatgctctccccacaatcgatgttctacaagctatgtatggccatccttcacctgaaaggcaaactttatagaggatgttttcataagggttcctgtccccaacttggtctgaaacaaacatgttgagttttctcttggccccgagaactgccttcaagaggtcctcgctgttgcttggcttgatcaaaattgactctaacatgttacccccatccaacagggctgcccctgccttcacggcagcaccaagactaaagttatagccagaaatgttgatgctggactgctgttcagtgatgacccccagaactgggtgcttgtctttcagcctttcaagatcattaagatttggatacttgactgtgtaaagcaagccaaggtctgtgagcgcttgtacaacgtcattgagcggagtctgtgactgtttggccatacaagccatagttagacttggcattgtgccaaattgattgttcaaaagtgatgagtctttcacatcccaaactcttaccacaccacttgcaccctgctgaggctttctcatcccaactatctgtaggatctgagatctttggtctagttgctgtgttgttaagttccccatatatacccctgaagcctggggcctttcagacctcatgatcttggccttcagcttctcaaggtcagccgcaagagacatcagttcttctgcactgagcctccccactttcaaaacattcttctttgatgttgactttaaatccacaagagaatgtacagtctggttgagacttctgagtctctgtaggtctttgtcatctctcttttccttcctcatgatcctctgaacattgctgacctcagagaagtccaacccattcagaaggttggttgcatccttaatgacagcagccttcacatctgatgtgaagctctgcaattctcttctcaatgcttgcgtccattggaagctcttaacttccttagacaaggacatcttgttgctcaatggtttctcaagacaaatgcgcaatcaaatgcctaggatccactgtgcg

SEQ ID NO: 6 - RNA, 7229 nt, Lymphocytic choriomeningitis mammarenavirus Viruses (LCMV)
  Lymphocytic choriomeningitis virus clone 13 segment L, complete sequence.-ACCESSION DQ361066-VERSION DQ361066.1-GI:86440167.-ssRNA viruses; ssRNA negative-strand viruses; Arenaviridae; Mammarenavirus
gcgcaccggggatcctaggcgtttagttgcgctgtttggttgcacaactttcttcgtgaggctgtcagaagtggacctggctgatagcgatgggtcaaggcaagtccagagaggagaaaggcaccaatagtacaaacagggccgaaatcctaccagataccacctatcttggccctttaagctgcaaatcttgctggcagaaatttgacagcttggtaagatgccatgaccactacctttgcaggcactgtttaaaccttctgctgtcagtatccgacaggtgtcctctttgtaaatatccattaccaaccagattgaagatatcaacagccccaagctctccacctccctacgaagagtaacaccgtccggccccggccccgacaaacagcccagcacaagggaaccgcacgtcacccaacgcacacagacacagcacccaacacagaacacgcacacacacacacacacacacccacacgcacgcgcccccaccaccggggggcgcccccccccggggggcggccccccgggagcccgggcggagccccacggagatgcccatcagtcgatgtcctcggccaccgacccgcccagccaatcgtcgcaggacctccccttgagtctaaacctgccccccactgtttcatacatcaaagtgctcctagatttgctaaaacaaagtctgcaatccttaaaggcgaaccagtctggcaaaagcgacagtggaatcagcagaatagatctgtctatacatagttcctggaggattacacttatctctgaacccaacaaatgttcaccagttctgaatcgatgcaggaagaggttcccaaggacatcactaatcttttcatagccctcaagtcctgctagaaagactttcatgtccttggtctccagcttcacaatgatattttggacaaggtttcttccttcaaaaagggcacccatctttacagtcagtggcacaggctcccactcaggtccaactctctcaaagtcaatagatctaatcccatccagtattcttttggagcccaacaactcaagctcaagagaatcaccaagtatcaagggatcttccatgtaatcctcaaactcttcagatctgatatcaaagacaccatcgttcaccttgaagacagagtctgtcctcagtaagtggaggcattcatccaacattcttctatctatctcacccttaaagaggtgagagcatgataaaagttcagccacacctggattctgtaattggcacctaaccaagaatatcaatgaaaatttccttaaacagtcagtattattctgattgtgcgtaaagtccactgaaattgaaaactccaataccccttttgtgtagttgagcatgtagtcccacagatcctttaaggatttaaatgcctttgggtttgtcaggccctgcctaatcaacatggcagcattacacacaacatctcccattcggtaagagaaccacccaaaaccaaactgcaaatcattcctaaacataggcctctccacatttttgttcaccacctttgagacaaatgattgaaaggggcccagtgcctcagcaccatcttcagatggcatcatttctttatgagggaaccatgaaaaattgcctaatgtcctggttgttgcaacaaattctcgaacaaatgattcaaaatacacctgttttaagaagttcttgcagacatccctcgtgctaacaacaaattcatcaaccagactggagtcagatcgctgatgagaattggcaaggtcagaaaacagaacagtgtaatgttcatcccttttccacttaacaacatgagaaatgagtgacaaggattctgagttaatatcaattaaaacacagaggtcaaggaatttaattctgggactccacctcatgttttttgagctcatgtcagacataaatggaagaagctgatcctcaaagatcttgggatatagccgcctcacagattgaatcacttggttcaaattcactttgtcctccagtagccttgagctctcaggctttcttgctacataatcacatgggtttaagtgcttaagagttaggttctcactgttattcttccctttggtcggttctgctaggacccaaacacccaactcaaaagagttgctcaatgaaatacaaatgtagtcccaaagaagaggccttaaaaggcatatatgatcacggtgggcttctggatgagactgtttgtcacaaatgtacagcgttataccatcccgattgcaaactcttgtcacatgatcatctgtggttagatcctcaagcagctttttgatatacagattttccctatttttgtttctcacacacctgcttcctagagttttgcaaaggcctataaagccagatgagatacaactctggaaagctgacttgttgattgcttctgacagcagcttctgtgcaccccttgtgaatttactacaaagtttgttctggagtgtcttgatcaatgatgggattctttcctcttggaaagtcatcactgatggataaaccaccttttgtcttaaaaccatccttaatgggaacatttcattcaaattcaaccagttaacatctgctaactgattcagatcttcttcaagaccgaggaggtctcccaattgaagaatggcctcctttttatctctgttaaataggtctaagaaaaattcttcattaaattcaccatttttgagcttatgatgcagtttccttacaagctttcttacaacctttgtttcattaggacacagttcctcaatgagtctttgtattctgtaacctctagaaccatccagccaatctttcacatcagtgttggtattcagtagaaatggatccaaagggaaattggcatactttaggaggtccagtgttctcctttggatactattaactagggagactgggacgccatttgcgatggcttgatctgcaattgtatctattgtttcacaaagttgatgtggctctttacacttgacattgtgtagcgctgcagatacaaactttgtgagaagagggacttcctccccccatacatagaatctagatttaaattctgcagcgaacctcccagccacactttttgggctgataaatttgtttaacaagccgctcagatgagattggaattccaacaggacaaggacttcctccggatcacttacaaccaggtcactcagcctcctatcaaataaagtgatctgatcatcacttgatgtgtaagcctctggtctttcgccaaagataacaccaatgcagtagttgatgaacctctcgctaagcaaaccatagaagtcagaagcattatgcaagattccctgccccatatcaataaggctggatatatgggatggcactatccccatttcaaaatattgtctgaaaattctctcagtaacagttgtttctgaacccctgagaagttttagcttcgacttgacatatgatttcatcattgcattcacaacaggaaaggggacctcgacaagcttatgcatgtgccaagttaacaaagtgctaacatgatctttcccggaacgcacatactggtcatcacctagtttgagattttgtagaaacattaagaacaaaaatgggcacatcattggtccccatttgctgtgatccatactatagtttaagaacccttcccgcacattgatagtcattgacaagattgcattttcaaattccttatcattgtttaaacaggagcctgaaaagaaacttgaaaaagactcaaaataatcttctattaaccttgtgaacatttttgtcctcaaatctccaatatagagttctctatttcccccaacctgctctttataagatagtgcaaatttcagccttccagagtcaggacctactgaggtgtatgatgttggtgattcttctgagtagaagcacagatttttcaaagcagcactcatacattgtgtcaacgacagagctttactaagggactcagaattactttccctctcactgattctcacgtcttcttccagtttgtcccagtcaaatttgaaattcaagccttgcctttgcatatgcctgtatttccctgagtacgcatttgcattcatttgcaacagaatcatcttcatgcaagaaaaccaatcattctcagaaaagaactttctacaaaggttttttgccatctcatcgaggccacactgatctttaatgactgaggtgaaatacaaaggtgacagctctgtggaaccctcaacagcctcacagataaatttcatgtcatcattggttagacatgatgggtcaaagtcttctactaaatggaaagatatttctgacaagataacttttcttaagtgagccatcttccctgttagaataagctgtaaatgatgtagtccttttgtatttgtaagtttttctccatctcctttgtcattggccctcctacctcttctgtaccgtgctattgtggtgttgaccttttcttcgagacttttgaagaagcttgtctcttcttctccatcaaaacatatttctgccaggttgtcttccgatctccctgtctcttctcccttggaaccgatgaccaatctagagactaacttggaaactttatattcatagtctgagtggctcaacttatacttttgttttcttacgaaactctccgtaatttgactcacagcactaacaagcaatttgttaaagtcatattccagaagtcgttctccatttagatgcttattaaccaccacacttttgttactagcaagatctaatgctgtcgcacatccagagttagtcatgggatctaggctgtttagcttcttctctcctttgaaaattaaagtgccgttgttaaatgaagacaccattaggctaaaggcttccagattaacacctggagttgtatgctgacagtcaatttctttactagtgaatctcttcatttgctcatagaacacacattcttcctcaggagtgattgcttccttggggttgacaaaaaaaccaaattgacttttgggctcaaagaacttttcaaaacattttatctgatctgttagcctgtcaggggtctcctttgtgatcaaatgacacaggtatgacacattcaacataaatttaaattttgcactcaacaacaccttctcaccagtaccaaaaatagtttttattaggaatctaagcagcttatacaccaccttctcagcaggtgtgatcagatcctccctcaacttatccattaatgatgtagatgaaaaatctgacactattgccatcaccaaatatctgacactctgtacctgcttttgatttctctttgttgggttggtgagcattagcaacaatagggtcctcagtgcaacctcaatgtcggtgagacagtctttcaaatcaggacatgatctaatccatgaaatcatgatgtctatcatattgtataagacctcatctgaaaaaattggtaaaaagaaccttttaggatctgcatagaaggaaattaaatgaccatccgggccttgtatggagtagcaccttgaagattctccagtcttctggtataataggtggtattcttcagagtccagttttattacttggcaaaacacttctttgcattctaccacttgatatctcacagaccctatttgattttgccttagtctagcaactgagctagttttcatactgtttgttaaggccagacaaacagatgataatcttctcaggctctgtatgttcttcagctgctctgtgctgggttggaaattgtaatcttcaaacttcgtataatacattatcgggtgagctccaattttcataaagttctcaaattcagtgaatggtatgtggcattcttgctcaaggtgttcagacagtccgtaatgctcgaaactcagtcccaccactaacaggcatttttgaatttttgcaatgaactcactaatagatgccctaaacaattcctcaaaagacacctttctaaacacctttgacttttttctattcctcaaaagtctaatgaactcctctttagtgctgtgaaagcttaccagcctatcattcacactactatagcaacaacccacccagtgtttatcattttttaaccctttgaatttcgactgttttatcaatgaggaaagacacaaaacatccagatttaacaactgtctccttctagtattcaacagtttcaaactcttgactttgtttaacatagagaggagcctctcatattcagtgctagtctcacttcccctttcgtgcccatgggtctctgcagttatgaatctcatcaaaggacaggattcgactgcctccctgcttaatgttaagatatcatcactatcagcaaggttttcatagagctcagagaattccttgatcaagccttcagggtttactttctgaaagtttctctttaatttcccactttctaaatctcttctaaacctgctgaaaagagagtttattccaaaaaccacatcatcacagctcatgttggggttgatgccttcgtggcacatcctcataatttcatcattgtgagttgacctcgcatctttcagaattttcatagagtccataccggagcgcttgtcgatagtagtcttcagggactcacagagtctaaaatattcagactcttcaaagactttctcattttggttagaatactccaaaagtttgaataaaaggtctctaaatttgaagtttgcccactctggcataaaactattatcataatcacaacgaccatctactattggaactaatgtgacacccgcaacagcaaggtcttccctgatgcatgccaatttgttagtgtcctctataaatttcttctcaaaactggctggagtgctcctaacaaaacactcaagaagaatgagagaattgtctatcagcttgtaaccatcaggaatgataagtggtagtcctgggcatacaattccagactccaccaaaattgtttccacagacttatcgtcgtggttgtgtgtgcagccactcttgtctgcactgtctatttcaatgcagcgtgacagcaacttgagtccctcaatcagaaccattctgggttccctttgtcccagaaagttgagtttctgccttgacaacctctcatcctgttctatatagtttaaacataactctctcaattctgagatgatttcatccattgcgcatcaaaaagcctaggatcctcggtgcg